European Patent Application EP 4 501 347 A1, published February 5, 2025. Title: Peptides for use in the treatment of Central Nervous System Disorders. Applicant: Prof. Wolf-Georg Forssmann. Application EP, filed August 2, 2023. The sequence listing filed with the application follows.

SEQUENCE LISTING (47 sequences)

SEQ ID NO: 1 - protein, 9 aa, Homo sapiens
VPQVSTPTL

SEQ ID NO: 2 - protein, 10 aa, Homo sapiens
KVPQVSTPTL

SEQ ID NO: 3 - protein, 11 aa, Homo sapiens
KKVPQVSTPTL

SEQ ID NO: 4 - protein, 12 aa, Homo sapiens
TKKVPQVSTPTL

SEQ ID NO: 5 - protein, 13 aa, Homo sapiens
YTKKVPQVSTPTL

SEQ ID NO: 6 - protein, 14 aa, Homo sapiens
RYTKKVPQVSTPTL

SEQ ID NO: 7 - protein, 15 aa, Homo sapiens
VRYTKKVPQVSTPTL

SEQ ID NO: 8 - protein, 16 aa, Homo sapiens
LVRYTKKVPQVSTPTL

SEQ ID NO: 9 - protein, 15 aa, Homo sapiens
LVRYTKKVPQVSTPT

SEQ ID NO: 10 - protein, 14 aa, Homo sapiens
LVRYTKKVPQVSTP

SEQ ID NO: 11 - protein, 13 aa, Homo sapiens
LVRYTKKVPQVST

SEQ ID NO: 12 - protein, 12 aa, Homo sapiens
LVRYTKKVPQVS

SEQ ID NO: 13 - protein, 11 aa, Homo sapiens
LVRYTKKVPQV

SEQ ID NO: 14 - protein, 10 aa, Homo sapiens
LVRYTKKVPQ

SEQ ID NO: 15 - protein, 9 aa, Homo sapiens
LVRYTKKVP

SEQ ID NO: 16 - protein, 8 aa, Homo sapiens
LVRYTKKV

SEQ ID NO: 17 - protein, 7 aa, Homo sapiens
LVRYTKK

SEQ ID NO: 18 - protein, 6 aa, Homo sapiens
LVRYTK

SEQ ID NO: 19 - protein, 8 aa, Homo sapiens
LLVRYTKK

SEQ ID NO: 20 - protein, 13 aa, Homo sapiens
LLVRYTKKVPQVS

SEQ ID NO: 21 - protein, 12 aa, synthetic construct
IVRYTKKVPQVS

SEQ ID NO: 22 - protein, 12 aa, synthetic construct
FVRYTKKVPQVS

SEQ ID NO: 23 - protein, 12 aa, synthetic construct
AVRYTKKVPQVS

SEQ ID NO: 24 - protein, 12 aa, synthetic construct
GVRYTKKVPQVS

SEQ ID NO: 25 - protein, 8 aa, synthetic construct
LVRYTKKA

SEQ ID NO: 26 - protein, 8 aa, synthetic construct
LVRYTKAV

SEQ ID NO: 27 - protein, 8 aa, synthetic construct
LVRYTAKV

SEQ ID NO: 28 - protein, 8 aa, synthetic construct
LVRYAKKV

SEQ ID NO: 29 - protein, 8 aa, synthetic construct
LVRATKKV

SEQ ID NO: 30 - protein, 8 aa, synthetic construct
LVAYTKKV

SEQ ID NO: 31 - protein, 8 aa, synthetic construct
LARYTKKV

SEQ ID NO: 32 - protein, 12 aa, synthetic construct
IVRWTKKVPQVS

SEQ ID NO: 33 - protein, 12 aa, synthetic construct
IVRWTCKVPQVS

SEQ ID NO: 34 - protein, 12 aa, synthetic construct
IVRWSKKVPCVS

SEQ ID NO: 35 - protein, 12 aa, synthetic construct
IVRWSKKVPQVS

SEQ ID NO: 36 - protein, 12 aa, synthetic construct
IMRWSRKMPCVS

SEQ ID NO: 37 - protein, 12 aa, synthetic construct
ILRWSRKLPCVS

SEQ ID NO: 38 - protein, 12 aa, synthetic construct
ILRWSRKMPCVS

SEQ ID NO: 39 - protein, 12 aa, synthetic construct
ILRWTRKMPCVS

SEQ ID NO: 40 - protein, 12 aa, synthetic construct
ILRWSRKMPCMS

SEQ ID NO: 41 - protein, 12 aa, synthetic construct
ILRWSRKFPCVS

SEQ ID NO: 42 - protein, 12 aa, synthetic construct
ILRWSRKMPCFS

SEQ ID NO: 43 - protein, 12 aa, synthetic construct
ILRWSRKMPQFS

SEQ ID NO: 44 - protein, 12 aa, synthetic construct
IVRWSKKMPQVS

SEQ ID NO: 45 - protein, 12 aa, synthetic construct
LVRYTQKAPQVS

SEQ ID NO: 46 - protein, 12 aa, synthetic construct
  VARIANT 4: note = X = Y or W
  VARIANT 5: note = X = T or S
  VARIANT 6: note = X = K, C, R, or Q
  VARIANT 8: note = X = V, M, L, F, or A
  VARIANT 10: note = X = Q or C
  VARIANT 11: note = X = V, M, or F
  VARIANT 2: note = X = V, M, or L
JXRXXXKXPXXS

SEQ ID NO: 47 - protein, 12 aa, synthetic construct
  VARIANT 5: note = X = T or S
  VARIANT 6: note = X = K or C
  VARIANT 10: note = X = Q or C
  VARIANT 4: note = X = Y or W
JVRXXXKVPXVS